European Patent Application EP 4 393 955 A1, published July 3, 2024. Title: 特异性结合CD47的抗体、其重组溶瘤病毒及其用途. Applicant: 上海鑫湾生物科技有限公司. The sequence listing filed with the application follows.

SEQUENCE LISTING (26 sequences)

SEQ ID NO: 1 - DNA, 1482 bp, synthetic construct
  source 1..1482: mol_type = other DNA
atggccctgcctgtgaccgccctcctcctgcctctcgccctgctcctccacgccgctagacccgaggtgcagctggtggagtctgggggaggcttggtccagcctggggggtccctgagactctcctgtgcagcctctggattcacctttagtggctatggcatgagctgggtccgccaggctccagggaaggggctggagtgggtggccaccataactagtggtggaacttacacctactatccagactctgtgaagggccgattcaccatctccagagacaacgccaagaactcactgtatctgcaaatgaacagcctgagagccgaggacacggctgtgtattactgtgcgagatccctcgcgggaaatgctatggactactggggccaaggaaccctggtcaccgtctcctcaggcggaggcggcagtggcgggggcgggtccggcggaggcgggagcgaaattgtgttgacacagtctccagccaccctgtctttgtctccaggggaaagagccaccctctcctgcagggccagtcagactattagcgactacttacactggtaccaacagaaacctggccaggctcccaggctcctcatcaaatttgcatcccaatccatttctggcatcccagccaggttcagtggcagtgggtctgggacagacttcactctcaccatcagcagcctagagcctgaagattttgcagtttattactgtcagaatggtcacggctttcctcggacgttcggccaagggaccaaggtggaaatcaaagagcccaaatcttgtgacaaaactcacacatgcccaccgtgcccagcacctgaactcctggggggaccgtcagtcttcctcttccccccaaaacccaaggacaccctcatgatctcccggacccctgaggtcacatgcgtggtggtggacgtgagccacgaagaccctgaggtcaagttcaactggtacgtggacggcgtggaggtgcataatgccaagacaaagccgcgggaggagcagtacaacagcacgtaccgtgtggtcagcgtcctcaccgtcctgcaccaggactggctgaatggcaaggagtacaagtgcaaggtctccaacaaagccctcccactccccgaggagaaaaccatctccaaagccaaagggcagccccgagaaccacaggtgtacaccctgcccccatcccgggatgagctgaccaagaaccaggtcagcctgacctgcctggtcaaaggcttctatcccagcgacatcgccgtggagtgggagagcaatgggcagccggagaacaactacaagaccacgcctcccgtgctggactccgacggctccttcttcctctacagcaagctcaccgtggacaagagcaggtggcagcaggggaacgtcttctcatgctccgtgatgcatgaggctctgcacaaccactacacgcagaagagcctctccctgtctccgggtaaatga

SEQ ID NO: 2 - protein, 493 aa, synthetic construct
MALPVTALLLPLALLLHAARPEVQLVESGGGLVQPGGSLRLSCAASGFTFSGYGMSWVRQAPGKGLEWVATITSGGTYTYYPDSVKGRFTISRDNAKNSLYLQMNSLRAEDTAVYYCARSLAGNAMDYWGQGTLVTVSSGGGGSGGGGSGGGGSEIVLTQSPATLSLSPGERATLSCRASQTISDYLHWYQQKPGQAPRLLIKFASQSISGIPARFSGSGSGTDFTLTISSLEPEDFAVYYCQNGHGFPRTFGQGTKVEIKEPKSCDKTHTCPPCPAPELLGGPSVFLFPPKPKDTLMISRTPEVTCVVVDVSHEDPEVKFNWYVDGVEVHNAKTKPREEQYNSTYRVVSVLTVLHQDWLNGKEYKCKVSNKALPLPEEKTISKAKGQPREPQVYTLPPSRDELTKNQVSLTCLVKGFYPSDIAVEWESNGQPENNYKTTPPVLDSDGSFFLYSKLTVDKSRWQQGNVFSCSVMHEALHNHYTQKSLSLSPGK

SEQ ID NO: 3 - DNA, 1026 bp, synthetic construct
  source 1..1026: mol_type = other DNA
gaggaggagctgcaggtgattcagcctgacaagtccgtatcagttgcagctggagagtcggccattctgcactgcactgtgacctccctgatccctgtggggcccatccagtggttcagaggagctggaccagcccgggaattaatctacaatcaaaaagaaggccacttcccccgggtaacaactgtttcagagtccacaaagagagaaaacatggacttttccatcagcatcagtaacatcaccccagcagatgccggcacctactactgtgtgaagttccggaaagggagccctgacacggagtttaagtctggagcaggcactgagctgtctgtgcgtgccaaaccctctgcccccgtggtatcgggccctgcggcgagggccacacctcagcacacagtgagcttcacctgcgagtcccacggcttctcacccagagacatcaccctgaaatggttcaaaaatgggaatgagctctcagacttccagaccaacgtggaccccgtaggagagagcgtgtcctacagcatccacagcacagccaaggtggtgctgacccgcgaggacgttcactctcaagtcatctgcgaggtggcccacgtcaccttgcagggggaccctcttcgtgggactgccaacttgtctgagaccatccgagttccacccaccttggaggttactcaacagcccgtgagggcagagaaccaggtgaatgtcacctgccaggtgaggaagttctacccccagagactacagctgacctggttggagaatggaaacgtgtcccggacagaaacggcctcaaccgttacagagaacaaggatggtacctacaactggatgagctggctcctggtgaatgtatctgcccacagggatgatgtgaagctcacctgccaggtggagcatgacgggcagccagcggtcagcaaaagccatgacctgaaggtctcagcccacccgaaggagcagggctcaaataccgccgctgagaacactggatctaatgaacggaacatctat

SEQ ID NO: 4 - protein, 342 aa, synthetic construct
EEELQVIQPDKSVSVAAGESAILHCTVTSLIPVGPIQWFRGAGPARELIYNQKEGHFPRVTTVSESTKRENMDFSISISNITPADAGTYYCVKFRKGSPDTEFKSGAGTELSVRAKPSAPVVSGPAARATPQHTVSFTCESHGFSPRDITLKWFKNGNELSDFQTNVDPVGESVSYSIHSTAKVVLTREDVHSQVICEVAHVTLQGDPLRGTANLSETIRVPPTLEVTQQPVRAENQVNVTCQVRKFYPQRLQLTWLENGNVSRTETASTVTENKDGTYNWMSWLLVNVSAHRDDVKLTCQVEHDGQPAVSKSHDLKVSAHPKEQGSNTAAENTGSNERNIY

SEQ ID NO: 5 - protein, 103 aa, synthetic construct
DIQMTQSPSSLSASVGDRVTITCRASQSITKSLNWYQQKPGKAPRLLIRVASTLQSGVPSRFSGSGSGTDFTLTISSLQPEDFATYYCQHSYSFGQGTKLEIT

SEQ ID NO: 6 - DNA, 309 bp, synthetic construct
  source 1..309: mol_type = other DNA
gacatccagatgacacagtctcctagctccctgtccgcctccgtgggcgaccgggtgaccattacatgccgcgcctctcagtctattaccaagagcctcaactggtatcagcagaagcccggcaaggccccaaggctgctgattagagtggcctctacactgcaatctggcgtgcctagcaggttcagcggctctggctccggcaccgacttcaccctgacaatttcttccctacagcccgaggacttcgccacatactactgccagcactcttactccttcggccagggcacaaagctagaaatcacc

SEQ ID NO: 7 - protein, 103 aa, synthetic construct
DIQMTQSPSTLSASVGDRVTITCRASQSISNWLAWYQQKPGEAPKLLIYKASNLESGVPSRFSGSGSGTEFTLTISSLQPDDFATYYCQQFGTFGQGTKVEIK

SEQ ID NO: 8 - DNA, 309 bp, synthetic construct
  source 1..309: mol_type = other DNA
gacattcagatgacacagtccccatccaccctgagcgcctccgtgggcgacagagtgaccattacatgccgcgcctctcagtctatttccaactggctcgcctggtatcagcagaagccaggcgaggcccctaagctgctgatttacaaggcctctaacttggagtctggcgtgccatctaggttctccggcagcggctccggcaccgagttcacactcacaattagctctttacaacccgacgacttcgccacatactactgccagcagttcggcaccttcggccagggcacaaaggtggagatcaag

SEQ ID NO: 9 - protein, 118 aa, synthetic construct
EVQLVESGGGLVQPGGSLRLSCAASGFTFSGYGMSWVRQAPGKGLEWVATITSGGTYTYYPDSVKGRFTISRDNAKNSLYLQMNSLRAEDTAVYYCARSLAGNAMDYWGQGTLVTVSS

SEQ ID NO: 10 - DNA, 354 bp, synthetic construct
  source 1..354: mol_type = other DNA
gaggtgcagctggtggagtctggcggcggcctcgtgcagcctggcggctccctgagactgtcctgcgccgcctctggcttcacattctccggctacggcatgtcttgggtgagacaggccccaggcaagggcctagagtgggtggccacaattacatccggcggcacatacacctactaccccgacagcgtgaagggcagattcaccatttcccgcgacaacgccaagaactctctgtacctccagatgaacagcctgagagccgaggacaccgccgtgtactactgcgcccggtcactcgccggcaacgctatggactactggggccagggcacactcgtgaccgtgtctagc

SEQ ID NO: 11 - protein, 11 aa, synthetic construct
RASQSITKSLN

SEQ ID NO: 12 - protein, 7 aa, synthetic construct
VASTLQS

SEQ ID NO: 13 - protein, 5 aa, synthetic construct
QHSYS

SEQ ID NO: 14 - protein, 11 aa, synthetic construct
RASQSISNWLA

SEQ ID NO: 15 - protein, 7 aa, synthetic construct
KASNLES

SEQ ID NO: 16 - protein, 5 aa, synthetic construct
QQFGT

SEQ ID NO: 17 - protein, 5 aa, synthetic construct
GYGMS

SEQ ID NO: 18 - protein, 17 aa, synthetic construct
TITSGGTYTYYPDSVKG

SEQ ID NO: 19 - protein, 9 aa, synthetic construct
SLAGNAMDY

SEQ ID NO: 20 - DNA, 37 bp, synthetic construct
  source 1..37: mol_type = other DNA
gtaccaggcctagtactatggagaggacccttgtctg

SEQ ID NO: 21 - DNA, 36 bp, synthetic construct
  source 1..36: mol_type = other DNA
aataagctcgaagtcgacctaggagagatgctgatg

SEQ ID NO: 22 - protein, 11 aa, synthetic construct
RAGQPLNNYLN

SEQ ID NO: 23 - protein, 7 aa, synthetic construct
AASTLQS

SEQ ID NO: 24 - protein, 5 aa, synthetic construct
QHRVT

SEQ ID NO: 25 - protein, 103 aa, synthetic construct
DIQMTQSPSSLSASVGDRVTITCRAGQPLNNYLNWYQQKPGKPPRLLIYAASTLQSGVPSRFSGSGSGTDFTLTISGLQSEDFASYFCQHRVTFGPGTKVDVR

SEQ ID NO: 26 - DNA, 309 bp, synthetic construct
  source 1..309: mol_type = other DNA
gacattcagatgacacagtccccatctagcgtgtctgcctccgtgggcgaccgggtgacaattacatgccgcgcctctcagggcattagctcacggctcgcctggtatcagcagaagcctggcaaggcccctaagctgctgatttacgccgcctcttccctccagagcggcgtgccatctaggttctctggctccggctctggcaccgacttcacactgaccatttcttcccttcaacccgaggacttcgccacatactactgccagcaggccaactccttcggcggcggcacaaaggtggagatcaag